European Patent Application EP 4 807 005 A1, published September 16, 2026. Title: 標的分子特異的な機能性タンパク質制御システム. Applicant: 国立大学法人京都大学. Application WO. The sequence listing filed with the application follows.

SEQUENCE LISTING (42 sequences)

SEQ ID NO: 1 - protein, 108 aa, synthetic construct
  REGION 1..108: note = humanized Trastuzumab VL
DIQMTQSPSSLSASVGDRVTITCRASQDVNTAVAWYQQKPGKAPKLLIYSASFLYSGVPSRFSGSGSGTDFTLTISSLQPEDFATYYCQQHYTTPPTFGQGTKVEIKR

SEQ ID NO: 2 - protein, 120 aa, synthetic construct
  REGION 1..120: note = humanized Trastuzumab VH
EVQLLESGGGLVQPGGSLRLSCAASGFNIKDTYIHWVRQAPGKGLEWVARIYPTNGYTRYADSVKGRFTISRDNSKNTLYLQMNSLRAEDTAVYYCSRWGGDGFYAMDYWGQGTLVTVSS

SEQ ID NO: 3 - protein, 24 aa, synthetic construct
  REGION 1..24: note = humanized Trastuzumab VL FR1
DIQMTQSPSSLSASVGDRVTITCR

SEQ ID NO: 4 - protein, 13 aa, synthetic construct
  REGION 1..13: note = humanized Trastuzumab VL FR 2
WYQQKPGKAPKLL

SEQ ID NO: 5 - protein, 31 aa, synthetic construct
  REGION 1..31: note = humanized Trastuzumab VL FR 3
GVPSRFSGSGSGTDFTLTISSLQPEDFATYY

SEQ ID NO: 6 - protein, 11 aa, synthetic construct
  REGION 1..11: note = humanized Trastuzumab VL FR 4
FGQGTKVEIKR

SEQ ID NO: 7 - protein, 26 aa, synthetic construct
  REGION 1..26: note = humanized Trastuzumab VH FR 1
EVQLLESGGGLVQPGGSLRLSCAASG

SEQ ID NO: 8 - protein, 12 aa, synthetic construct
  REGION 1..12: note = humanized Trastuzumab VH FR 2
WVRQAPGKGLEW

SEQ ID NO: 9 - protein, 37 aa, synthetic construct
  REGION 1..37: note = humanized Trastuzumab VH FR 3
YADSVKGRFTISRDNSKNTLYLQMNSLRAEDTAVYYC

SEQ ID NO: 10 - protein, 13 aa, synthetic construct
  REGION 1..13: note = humanized Trastuzumab VH FR 4
DYWGQGTLVTVSS

SEQ ID NO: 11 - protein, 37 aa, synthetic construct
  REGION 1..37: note = humanized Trastuzumab VH FR 3-2
YADSVKGRFTISADNSKNTLYLQMNSLRAEDTAVYYC

SEQ ID NO: 12 - protein, 179 aa, synthetic construct
  REGION 1..179: note = T7N (d5-19) (N-terminal T7 RNAP fragment)
MNTINIAKNDFSDIELAAIPLNTLADHYGERSARGQLALEHESYEMGEARFRKMFECQLKAGKVADNAAAKPLITTLLPKMIARINDWFEEVKAKRGRRPTAFKFLKEIKPEAVAYITIKTSLACLTSADNTTVQAVASAIGRTIEDEARFGRIRDLEAKHFKKNVEEQLNKRVGHVYK

SEQ ID NO: 13 - protein, 704 aa, synthetic construct
  REGION 1..704: note = T7C (C-terminal T7 RNAP fragment)
KAFMQVVEADMLSKGLLGGEAWSSWHKEDSIHVGVRCIEMLIESTGMVSLHRQNAGVVGQDSETIELAPEYAEAIATRAGALAGISPMFQPCVVPPKPWTGITGGGYWANGRRPLALVRTHSKKALMRYEDVYMPEVYKAINIAQNTAWKINKKVLAVANVITKWKHCPVEDIPAIEREELPMKPEDIDMNPEALTAWKRAAAAVYRKDKARKSRRISLEFMLEQANKFANHKAIWFPYNMDWRGRVYAVSMFNPQGNDMTKGLLTLAKGKPIGKEGYYWLKIHGANCAGVDKVPFPERIKFIEENHENIMACAKSPLENTWWAEQDSPFCFLAFCFEYAGVQHHGLSYNCSLPLAFDGSCSGIQHFSAMLRDEVGGRAVNLLPSETVQDIYGIVAKKVNEILQADAINGTDNEVVTVTDENTGEISEKVKLGTKALAGQWLAYGVTRSVTKRSVMTLAYGSKEFGFRQQVLEDTIQPAIDSGKGLMFTQPNQAAGYMAKLIWESVSVTVVAAVEAMNWLKSAAKLLAAEVKDKKTGEILRKRCAVHWVTPDGFPVWQEYKKPIQTRLNLMFLGQFRLQPTINTNKDSEIDAHKQESGIAPNFVHSQDGSHLRKTVVWAHEKYGIESFALIHDSFGTIPADAANLFKAVRETMVDTYESCDVLADFYDQFADQLHESQLDKMPALPAKGNLNLRDILESDFAFA

SEQ ID NO: 14 - protein, 704 aa, synthetic construct
  REGION 1..704: note = CGG RNAPc (C-terminal CGG RNAP fragment)
KAFMQVVEADMLSKGLLGGEAWSSWHKEDSIHVGVRCIEMLIESTGMVSLHRQNAGVVGQDSETIELAPEYAEAIATRAGALAGISPMFQPCVVPPKPWTGITGGGYWANGRRPLALVRTHSKKALMRYEDVYMPEVYKAINIAQNTAWKINKKVLAVANVITKWKHCPVEDIPAIEREELPMKPEDIDMNPEALTAWKRAAAAVYRKDKARKSRRISLEFMLEQANKFANHKAIWFPYNMDWRGRVYAVSMFNPQGNDMTKGLLTLAKGKPIGKEGYYWLKIHGANCAGVDKVPFPERIKFIEENHENIMACAKSPLENTWWAEQDSPFCFLAFCFEYAGVQHHGLSYNCSLPLAFDGSCSGIQHFSAMLRDEVGGRAVNLLPSETVQDIYGIVAKKVNEILQADAINGTDNEVVTVTDENTGEISEKVKLGTKALAGQWLAYGVTRSVTKRSVMTLAYGSKEFGFRQQVLEDTIQPAIDSGKGLMFTQPNQAAGYMAKLIWESVSVTVVAAVEAMNWLKSAAKLLAAEVKDKKTGEILRKRCAVHWVTPDGFPVWQEYKKPIKTRVHIMFLGQFEMQPTINTNKDSEIDARKQVSGIAPNFVHSQDGSHLRKTVVWAHEKYGIESFALIHDSFGTIPADAANLFKAVRETMVDTYESCDVLADFYDQFADQLHESQLDKMPALPAKGNLNLRDILESDFAFA

SEQ ID NO: 15 - protein, 883 aa, synthetic construct
  REGION 1..883: note = CGG RNAP
MNTINIAKNDFSDIELAAIPFNTLADHYGERLAREQLALEHESYEMGEARFRKMFERQLKAGEVADNAAAKPLITTLLPKMIARINDWFEEVKAKRGKRPTAFQFLQEIKPEAVAYITIKTTLACLTSADNTTVQAVASAIGRAIEDEARFGRIRDLEAKHFKKNVEEQLNKRVGHVYKKAFMQVVEADMLSKGLLGGEAWSSWHKEDSIHVGVRCIEMLIESTGMVSLHRQNAGVVGQDSETIELAPEYAEAIATRAGALAGISPMFQPCVVPPKPWTGITGGGYWANGRRPLALVRTHSKKALMRYEDVYMPEVYKAINIAQNTAWKINKKVLAVANVITKWKHCPVEDIPAIEREELPMKPEDIDMNPEALTAWKRAAAAVYRKDKARKSRRISLEFMLEQANKFANHKAIWFPYNMDWRGRVYAVSMFNPQGNDMTKGLLTLAKGKPIGKEGYYWLKIHGANCAGVDKVPFPERIKFIEENHENIMACAKSPLENTWWAEQDSPFCFLAFCFEYAGVQHHGLSYNCSLPLAFDGSCSGIQHFSAMLRDEVGGRAVNLLPSETVQDIYGIVAKKVNEILQADAINGTDNEVVTVTDENTGEISEKVKLGTKALAGQWLAYGVTRSVTKRSVMTLAYGSKEFGFRQQVLEDTIQPAIDSGKGLMFTQPNQAAGYMAKLIWESVSVTVVAAVEAMNWLKSAAKLLAAEVKDKKTGEILRKRCAVHWVTPDGFPVWQEYKKPIKTRVHIMFLGQFEMQPTINTNKDSEIDARKQVSGIAPNFVHSQDGSHLRKTVVWAHEKYGIESFALIHDSFGTIPADAANLFKAVRETMVDTYESCDVLADFYDQFADQLHESQLDKMPALPAKGNLNLRDILESDFAFA

SEQ ID NO: 16 - protein, 111 aa, synthetic construct
  REGION 1..111: note = VL domain (Anti-GCN4 antibody)
DIVMTQSPSSLSASVGDRVTITCRSSTGAVTTSNYASWVQEKPGKLFKGLIGGTNNRAPGVPSRFSGSLIGDKATLTISSLQPEDFATYFCALWYSNHWVFGQGTKVELKR

SEQ ID NO: 17 - protein, 113 aa, synthetic construct
  REGION 1..113: note = VH domain (Anti-GCN4 antibody)
EVKLLESGGGLVQPGGSLKLSCAVSGFSLTDYGVNWVRQAPGRGLEWIGVIWGDGITDYNSALKDRFIISKDNGKNTVYLQMSKVRSDDTALYYCVTGLFDYWGQGTLVTVSS

SEQ ID NO: 18 - protein, 113 aa, synthetic construct
  REGION 1..113: note = VH domain (WT), (Anti-GCN4 antibody, omega-grafted framework)
EVKLLESGGGLVQPGGSLKLSCAVSGFSLTDYGVNWVRQAPGRGLEWIGVIWGDGITDYNSALKDRFIISKDDCENTVYLQMSKVRSDDTALYYCVTGLFDYWGQGTLVTVSS

SEQ ID NO: 19 - protein, 113 aa, synthetic construct
  REGION 1..113: note = VH domain (GLW), (Anti-GCN4 antibody, omega-grafted framework)
EVKLLESGGGLVQPGGSLKLSCAVSGFSLTDYGVNWVRQAPGRGLEWIGVIWGDGITDYNSALKDRFIISKDDCENTVYLQMSKVRSDDTALYYCVTGLWDYWGQGTLVTVSS

SEQ ID NO: 20 - protein, 113 aa, synthetic construct
  REGION 1..113: note = VH domain (ALF), (Anti-GCN4 antibody, omega-grafted framework)
EVKLLESGGGLVQPGGSLKLSCAVSGFSLTDYGVNWVRQAPGRGLEWIGVIWGDGITDYNSALKDRFIISKDDCENTVYLQMSKVRSDDTALYYCVTALFDYWGQGTLVTVSS

SEQ ID NO: 21 - protein, 113 aa, synthetic construct
  REGION 1..113: note = VH domain (GFA), (Anti-GCN4 antibody, omega-grafted framework)
EVKLLESGGGLVQPGGSLKLSCAVSGFSLTDYGVNWVRQAPGRGLEWIGVIWGDGITDYNSALKDRFIISKDDCENTVYLQMSKVRSDDTALYYCVTGFADYWGQGTLVTVSS

SEQ ID NO: 22 - protein, 113 aa, synthetic construct
  REGION 1..113: note = VL domain (Anti-FLAG antibody, trastuzumab framework)
DIQMTQSPSSLSASVGDRVTITCRSSQSIVHRNGNTYLEWYQQKPGKAPKLLIYKVSNRFSGVPSRFSGSGSGTDFTLTISSLQPEDFATYYCFQGSHVPYTFGQGTKVEIKR

SEQ ID NO: 23 - protein, 117 aa, synthetic construct
  REGION 1..117: note = VH domain (Anti-FLAG antibody, trastuzumab framework)
EVQLLESGGGLVQPGGSLRLSCAASGYSFTTYTIHWVRQAPGKGLEWIGYINPSSGYAAYADSVKGRFTISRDNSKNTLYLQMNSLRAEDTAVYYCAREKFYGYDYWGQGTLVTVSS

SEQ ID NO: 24 - protein, 108 aa, synthetic construct
  REGION 1..108: note = VL domain (Anti-EGFP antibody)
DIQMTQSPSSLSASVGDRVTITCRASQSISSYLNWYQQKPGKAPKLLIYYASYLQSGVPSRFSGSGSGTDFTLTISSLQPEDFATYYCQQTAAGPSTFGQGTKVEIKR

SEQ ID NO: 25 - protein, 116 aa, synthetic construct
  REGION 1..116: note = VH domain (Anti-EGFP antibody)
EVQLLESGGGLVQPGGSLRLSCAASGFTFSSYAMSWVRQAPGKGLEWVSYISGTGNTTAYADSVKGRFTISRDNSKNTLYLQMNSLRAEDTAVYYCAKDTNYFDYWGQGTLVTVSS

SEQ ID NO: 26 - protein, 108 aa, synthetic construct
  REGION 1..108: note = VL domain (Anti-HCV IRES RNA antibody)
DIQMTQSPSSLSASVGDRVTITCRASQSVSSAVAWYQQKPGKAPKLLIYSASSLYSGVPSRFSGSGSGTDFTLTISSLQPEDFATYYCQQSSYYPSTFGQGTKVEIKR

SEQ ID NO: 27 - protein, 122 aa, synthetic construct
  REGION 1..122: note = VH domain (Anti-HCV IRES RNA antibody)
EVQLLESGGGLVQPGGSLRLSCAASGFYISSYSIHWVRQAPGKGLEWVASIYPSYGYTSYADSVKGRFTISADNSKNTLYLQMNSLRAEDTAVYYCARRYRSYYSRYGFDYWGQGTLVTVSS

SEQ ID NO: 28 - protein, 113 aa, synthetic construct
  REGION 1..113: note = VL domain (Anti-Fluorescein antibody)
DIQMTQSPSSLSASVGDRVTITCRSSQSLVHSNGNTYLRWYQQKPGKAPKLLIYKVSNRVSGVPSRFSGSGSGTDFTLTISSLQPEDFATYYCSQSTHVPWTFGQGTKVEIKR

SEQ ID NO: 29 - protein, 118 aa, synthetic construct
  REGION 1..118: note = VH domain (Anti-Fluorescein antibody)
EVQLLESGGGLVQPGGSLRLSCAASGFTFGHYWMNWVRQAPGKGLEWVAQFRNKPYNYETYYADSVKGRFTISRDNSKNTLYLQMNSLRAEDTAVYYCTGASYGMEYWGQGTLVTVSS

SEQ ID NO: 30 - protein, 111 aa, synthetic construct
  REGION 1..111: note = VL domain (Anti-Hsp70 antibody)
DIQMTQSPSSLSASVGDRVTITCRSSTGAVTTSNYANWYQQKPGKAPKLLIGGTNNRAPGVPSRFSGSGSGTDFTLTISSLQPEDFATYYCALWYSNHLVFGQGTKVEIKR

SEQ ID NO: 31 - protein, 117 aa, synthetic construct
  REGION 1..117: note = VH domain (Anti-Hsp70 antibody)
EVQLLESGGGLVQPGGSLRLSCAASGFSLSRNSVHWVRQAPGKGLEWLGMIWGGGSTDYADSVKGRFTISRDNSKNTLYLQMNSLRAEDTAVYYCARNGGYDVFDYWGQGTLVTVSS

SEQ ID NO: 32 - protein, 19 aa, synthetic construct
  REGION 1..19: note = GCN4 peptide
EELLSKNYHLENEVARLKK

SEQ ID NO: 33 - protein, 8 aa, synthetic construct
  REGION 1..8: note = 1xFLAG peptide
DYKDDDDK

SEQ ID NO: 34 - protein, 22 aa, synthetic construct
  REGION 1..22: note = 3xFLAG peptide
DYKDHDGDYKDHDIDYKDDDDK

SEQ ID NO: 35 - DNA, 20 bp, synthetic construct
  misc_feature 1..20: note = T7 promoter
  source 1..20: mol_type = other DNA
taatacgactcactataggg

SEQ ID NO: 36 - DNA, 20 bp, synthetic construct
  misc_feature 1..20: note = CGG promoter
  source 1..20: mol_type = other DNA
taataccggtcactataggg

SEQ ID NO: 37 - DNA, 333 bp, synthetic construct
  misc_feature 1..333: note = HCV IRES
  source 1..333: mol_type = other DNA
ctcccctgtgaggaactactgtcttcacgcagaaagcgtctagccatggcgttagtatgagagtcgtgcagcctccaggaccccccctcccgggagagccatagtggtctgcggaaccggtgagtacaccggaattgccaggacgaccgggtcctttcttggatcaacccgctcaatgcctggagatttgggcgtgcccccgcaagactgctagccgagtagtgttgggtcgcgaaaggccttgtggtactgcctgatagggtgcttgcgagtgccccgggaggtctcgtagaccgtgcaccatgagcacgaatcctaaacctcaaagaaaaa

SEQ ID NO: 38 - DNA, 95 bp, synthetic construct
  misc_feature 1..95: note = EGFP-targeting gRNA
  source 1..95: mol_type = other DNA
gcacgggcagcttgccgggttttagagctagaaatagcaagttaaaataaggctagtccgttatcaacttgaaaaagtggcaccgagtcggtgct

SEQ ID NO: 39 - DNA, 717 bp, synthetic construct
  misc_feature 1..717: note = EGFP (gRNA target sequence is underlined)
  source 1..717: mol_type = other DNA
atggtgagcaagggcgaggagctgttcaccggggtggtgcccatcctggtcgagctggacggcgacgtaaacggccacaagttcagcgtgtccggcgagggcgagggcgatgccacctacggcaagctgaccctgaagttcatctgcaccaccggcaagctgcccgtgccctggcccaccctcgtgaccaccctgacctacggcgtgcagtgcttcagccgctaccccgaccacatgaagcagcacgacttcttcaagtccgccatgcccgaaggctacgtccaggagcgcaccatcttcttcaaggacgacggcaactacaagacccgcgccgaggtgaagttcgagggcgacaccctggtgaaccgcatcgagctgaagggcatcgacttcaaggaggacggcaacatcctggggcacaagctggagtacaactacaacagccacaacgtctatatcatggccgacaagcagaagaacggcatcaaggtgaacttcaagatccgccacaacatcgaggacggcagcgtgcagctcgccgaccactaccagcagaacacccccatcggcgacggccccgtgctgctgcccgacaaccactacctgagcacccagtccgccctgagcaaagaccccaacgagaagcgcgatcacatggtcctgctggagttcgtgaccgccgccgggatcactctcggcatggacgagctgtacaag

SEQ ID NO: 40 - DNA, 221 bp, synthetic construct
  misc_feature 1..221: note = Human HSP70 promoter
  source 1..221: mol_type = other DNA
ccctgtcccctccagtgaatcccagaagactctggagagttctgagcagggggcggcactctggcctctgattggtccaaggaaggctggggggcaggacgggaggcgaaaaccctggaatattcccgacctggcagcctcatcgagctcggtgattggctcagaagggaaaaggcgggtctccgtgacgacttataaaagcccaggggcaagcggtccgg

SEQ ID NO: 41 - protein, 108 aa, synthetic construct
DIQMTQSPSSLSASVGDRVTITCRASQDVNTAVAWYQQKPGKAPKLLIYSASFLYSGVPSRFSGSRSGTDFTLTISSLQPEDFATYYCQQHYTTPPTFGQGTKVEIKR

SEQ ID NO: 42 - protein, 120 aa, synthetic construct [sequence omitted]